European Patent Application EP 4 491 710 A1, published January 15, 2025. Title: A microorganism producing O-acetyl homoserine and a method for producing O-acetyl homoserine or L-methionine using the same. Applicant: CJ CheilJedang Corporation. The sequence listing filed with the application follows.

SEQUENCE LISTING (28 sequences)

SEQ ID NO: 1 - protein, 179 aa, Corynebacterium glutamicum
MVERDFTIRPIREGDFPQVRDIYELGLETGHATYETSGPTWDQFSQSKIMDTVMVAVENNDPDFILGWVSAAPISSRQVFHGVVEDSIYIHPQGQGRGIGGALLDALITYCESNGIWSIHSWIFPENLGSAKLHESKGFVKVGTMHQMARMPYGEMEGQWRDCDLWECLLSVPEQAQSS

SEQ ID NO: 2 - DNA, 540 bp, Corynebacterium glutamicum
  source 1..540: mol_type = genomic DNA
atggttgaaagagacttcactatccgaccaatccgcgagggtgatttccctcaggtgagggacatctacgaattgggcctggagacgggacatgcgacttatgagacttctggtcccacgtgggaccagttctcccaatctaaaatcatggataccgtcatggtggcggtagaaaacaacgacccggacttcatcctcggatgggtgtctgctgctccaatttcaagccgacaggttttccatggagtggtggaagattccatctatatccacccccagggccaaggccgaggaatcggcggcgctttgctcgacgcccttatcacctactgcgaaagcaacggcatctggtcgatccactcctggatcttcccggaaaacctcggttctgcgaaactgcatgaatcgaagggcttcgtgaaggtgggcaccatgcaccaaatggcaaggatgccctacggcgagatggaaggacaatggcgcgattgtgatctgtgggagtgcctcttatccgttccagagcaagctcaaagttcctaa

SEQ ID NO: 3 - DNA, 40 bp, synthetic construct
  misc_feature 1..40: note = 0959 _del up F
  source 1..40: mol_type = other DNA
tgaattcgagctcggtacccatccacagacggtcatcgtg

SEQ ID NO: 4 - DNA, 33 bp, synthetic construct
  misc_feature 1..33: note = 0959 _del up R
  source 1..33: mol_type = other DNA
tttggtggatatccatgcacgcaattgtcctgg

SEQ ID NO: 5 - DNA, 33 bp, synthetic construct
  misc_feature 1..33: note = 0959 _del down F
  source 1..33: mol_type = other DNA
gtgcatggatatccaccaaatggcaaggatgcc

SEQ ID NO: 6 - DNA, 40 bp, synthetic construct
  misc_feature 1..40: note = 0959 _del down R
  source 1..40: mol_type = other DNA
gtcgactctagaggatccccgcagagatcgttgattcaat

SEQ ID NO: 7 - DNA, 5803 bp, synthetic construct
  misc_feature 1..5803: note = pDCM2
  source 1..5803: mol_type = other DNA
gttcgcttgctgtccataaaaccgcccagtctagctatcgccatgtaagcccactgcaagctacctgctttctctttgcgcttgcgttttcccttgtccagatagcccagtagctgacattcatccggggtcagcaccgtttctgcggactggctttctacgtgttccgcttcctttagcagcccttgcgccctgagtgcttgcggcagcgtgaagctagcttttatcgccattcgccattcaggctgcgcaactgttgggaagggcgatcggtgcgggcctcttcgctattacgccagctggcgaaagggggatgtgctgcaaggcgattaagttgggtaacgccagggttttcccagtcacgacgttgtaaaacgacggccagtgaattcgagctcggtacccggggatcctctagagtcgacctgcaggcatgcaagcttggcgtaatcatggtcatagctgtttcctgtgtgaaattgttatccgctcacaattccacacaacatacgagccggaagcataaagtgtaaagcctggggtgcctaatgagtgagctaactcacattaattgcgttgcgctcactgcccgctttccagtcgggaaacctgtcgtgccagctgcattaatgaatcggccaacgcgcggggagaggcggtttgcgtattgggcgctcttccgcttcctcgctcactgactcgctgcgctcggtcgttcggctgcggcgagcggtatcagctcactcaaaggcggtaatacggttatccacagaatcaggggataacgcaggaaagaacatgtgagcaaaaggccagcaaaaggccaggaaccgtaaaaaggccgcgttgctggcgtttttccataggctccgcccccctgacgagcatcacaaaaatcgacgctcaagtcagaggtggcgaaacccgacaggactataaagataccaggcgtttccccctggaagctccctcgtgcgctctcctgttccgaccctgccgcttaccggatacctgtccgcctttctcccttcgggaagcgtggcgctttctcaatgctcacgctgtaggtatctcagttcggtgtaggtcgttcgctccaagctgggctgtgtgcacgaaccccccgttcagcccgaccgctgcgccttatccggtaactatcgtcttgagtccaacccggtaagacacgacttatcgccactggcagcagccactggtaacaggattagcagagcgaggtatgtaggcggtgctacagagttcttgaagtggtggcctaactacggctacactagaaggacagtatttggtatctgcgctctgctgaagccagttaccttcggaaaaagagttggtagctcttgatccggcaaacaaaccaccgctggtagcggtggtttttttgtttgcaagcagcagattacgcgcagaaaaaaaggatctcaagaagatcctttgatcttttctacggggtctgacgctcagtggaacgaaaactcacgttaagggattttggtcatgagattatcaaaaaggatcttcacctagatccttttggggtgggcgaagaactccagcatgagatccccgcgctggaggatcatccagccctgatagaaacagaagccactggagcacctcaaaaacaccatcatacactaaatcagtaagttggcagcatcacccgacgcactttgcgccgaataaatacctgtgacggaagatcacttcgcagaataaataaatcctggtgtccctgttgataccgggaagccctgggccaacttttggcgaaaatgagacgttgatcggcacgtaagaggttccaactttcaccataatgaaataagatcactaccgggcgtattttttgagttatcgagattttcaggagctgatagaaacagaagccactggagcacctcaaaaacaccatcatacactaaatcagtaagttggcagcatcacccgacgcactttgcgccgaataaatacctgtgacggaagatcacttcgcagaataaataaatcctggtgtccctgttgataccgggaagccctgggccaacttttggcgaaaatgagacgttgatcggcacgtaagaggttccaactttcaccataatgaaataagatcactaccgggcgtattttttgagttatcgagattttcaggagctctttggcatcgtctctcgcctgtcccctcagttcagtaatttcctgcatttgcctgtttccagtcggtagatattccacaaaacagcagggaagcagcgcttttccgctgcataaccctgcttcggggtcattatagcgattttttcggtatatccatcctttttcgcacgatatacaggattttgccaaagggttcgtgtagactttccttggtgtatccaacggcgtcagccgggcaggataggtgaagtaggcccacccgcgagcgggtgttccttcttcactgtcccttattcgcacctggcggtgctcaacgggaatcctgctctgcgaggctggccggctaccgccggcgtaacagatgagggcaagcggatggctgatgaaaccaagccaaccaggaagggcagcccacctatcaaggtgtactgccttccagacgaacgaagagcgattgaggaaaaggcggcggcggccggcatgagcctgtcggcctacctgctggccgtcggccagggctacaaaatcacgggcgtcgtggactatgagcacgtccgcgagggcgtcccggaaaacgattccgaagcccaacctttcatagaaggcggcggtggaatcgaaatctcgtgatggcaggttgggcgtcgcttggtcggtcatttcgaaaaaggttaggaatacggttagccatttgcctgcttttatatagttcantatgggattcacctttatgttgataagaaataaaagaaaatgccaataggatatcggcattttcttttgcgtttttatttgttaactgttaattgtccttgttcaaggatgctgtctttgacaacagatgttttcttgcctttgatgttcagcaggaagctcggcgcaaacgttgattgtttgtctgcgtagaatcctctgtttgtcatatagcttgtaatcacgacattgtttcctttcgcttgaggtacagcgaagtgtgagtaagtaaaggttacatcgttaggcggatcaagatccatttttaacacaaggccagttttgttcagcggcttgtatgggccagttaaagaattagaaacataaccaagcatgtaaatatcgttagacgtaatgccgtcaatcgtcatttttgatccgcgggagtcagtgaacaggtaccatttgccgttcattttaaagacgttcgcgcgttcaatttcatctgttactgtgttagatgcaatcagcggtttcatcacttttttcagtgtgtaatcatcgtttagctcaatcataccgagagcgccgtttgctaactcagccgtgcgttttttatcgctttgcagaagtttttgactttcttgacggaagaatgatgtgcttttgccatagtatgctttgttaaataaagattcttcgccttggtagccatcttcagttccagtgtttgcttcaaatactaagtatttgtggcctttatcttctacgtagtgaggatctctcagcgtatggttgtcgcctgagctgtagttgccttcatcgatgaactgctgtacattttgatacgtttttccgtcaccgtcaaagattgatttataatcctctacaccgttgatgttcaaagagctgtctgatgctgatacgttaacttgtgcagttgtcagtgtttgtttgccgtaatgtttaccggagaaatcagtgtagaataaacggatttttccgtcagatgtaaatgtggctgaacctgaccattcttgtgtttggtcttttaggatagaatcatttgcatcgaatttgtcgctgtctttaaagacgcggccagcgtttttccagctgtcaatagaagtttcgccgactttttgatagaacatgtaaatcgatgtgtcatccgcatttttaggatctccggctaatgcaaagacgatgtggtagccgtgatagtttgcgacagtgccgtcagcgttttgtaatggccagctgtcccaaacgtccaggccttttgcagaagagatatttttaattgtggacgaatcaaattcagaaacttgatatttttcatttttttgctgttcagggatttgcagcatatcatggcgtgtaatatgggaaatgccgtatgtttccttatatggcttttggttcgtttctttcgcaaacgcttgagttgcgcctcctgccagcagtgcggtagtaaaggttaatactgttgcttgttttgcaaactttttgatgttcatcgttcatgtctccttttttatgtactgtgttagcggtctgcttcttccagccctcctgtttgaagatggcaagttagttacgcacaataaaaaaagacctaaaatatgtaaggggtgacgccaaagtatacactttgccctttacacattttaggtcttgcctgctttatcagtaacaaacccgcgcgatttacttttcgacctcattctattagactctcgtttggattgcaactggtctattttcctcttttgtttgatagaaaatcataaaaggatttgcagactacgggcctaaagaactaaaaaatctatctgtttcttttcattctctgtattttttatagtttctgttgcatgggcataaagttgcctttttaatcacaattcagaaaatatcataatatctcatttcactaaataatagtgaacggcaggtatatgtgatgggttaaaaaggatcaccccagagtcccgctcagaagaactcgtcaagaaggcgatagaaggcgatgcgctgcgaatcgggagcggcgataccgtaaagcacgaggaagcggtcagcccattcgccgccaagctcttcagcaatatcacgggtagccaacgctatgtcctgatagcggtccgccacacccagccggccacagtcgatgaatccagaaaagcggccattttccaccatgatattcggcaagcaggcatcgccatgggtcacgacgagatcctcgccgtcgggcatccgcgccttgagcctggcgaacagttcggctggcgcgagcccctgatgctcttcgtccagatcatcctgatcgacaagaccggcttccatccgagtacgtgctcgctcgatgcgatgtttcgcttggtggtcgaatgggcaggtagccggatcaagcgtatgcagccgccgcattgcatcagccatgatggatactttctcggcaggagcaaggtgagatgacaggagatcctgccccggcacttcgcccaatagcagccagtcccttcccgcttcagtgacaacgtcgagacagctgcgcaaggaacgcccgtcgtggccagccacgatagccgcgctgcctcgtcttggagttcattcagggcaccggacaggtcggtcttgacaaaaagaaccgggcgcccctgcgctgacagccggaacacggcggcatcagagcagccgattgtctgttgtgcccagtcatagccgaatagcctctccacccaagcggccggagaacctgcgtgcaatccatcttgttcaatcatgcgaaacgatcctcatcctgtctcttgatcagatcttgatcccctgcgccatcagatccttggcggcaagaaagccatccagtttactttgcagggcttcccaaccttaccagagggcgccccagctggcaattccg

SEQ ID NO: 8 - DNA, 25 bp, synthetic construct
  misc_feature 1..25: note = 0959 _del F
  source 1..25: mol_type = other DNA
gtgaaaaaacactggcaaaacaagc

SEQ ID NO: 9 - DNA, 25 bp, synthetic construct
  misc_feature 1..25: note = 0959 _del R
  source 1..25: mol_type = other DNA
ataagaggcactcccacagatcaca

SEQ ID NO: 10 - protein, 418 aa, synthetic construct
  REGION 1..418: note = YjeH F351L
MSGLKQELGLAQGIGLLSTSLLGTGVFAVPALAALVAGNNSLWAWPVLIILVFPIAIVFAILGRHYPSAGGVAHFVGMAFGSRLERVTGWLFLSVIPVGLPAALQIAAGFGQAMFGWHSWQLLLAELGTLALVWYIGTRGASSSANLQTVIAGLIVALIVAIWWAGDIKPANIPFPAPGNIELTGLFAALSVMFWCFVGLEAFAHLASEFKNPERDFPRALMIGLLLAGLVYWGCTVVVLHFDAYGEKMAAAASLPKIVVQLFGVGALWIACVIGYLACFASLNIYIQSFARLVWSQAQHNPDHYLARLSSRHIPNNALNAVLGCCVVSTLVIHALEINLDALIIYANGILIMIYLLCMLAGCKLLQGRYRLLAVVGGLLCVLLLAMVGWKSLYALIMLAGLWLLLPKRKTPENGITT

SEQ ID NO: 11 - DNA, 1161 bp, unidentified
  misc_feature 1..1161: note = Corynebacterium glutamicum metB
  source 1..1161: mol_type = genomic DNA
ttgtcttttgacccaaacacccagggtttctccactgcatcgattcacgctgggtatgagccagacgactactacggttcgattaacaccccaatctatgcctccaccaccttcgcgcagaacgctccaaacgaactgcgcaaaggctacgagtacacccgtgtgggcaaccccaccatcgtggcattagagcagaccgtcgcagcactcgaaggcgcaaagtatggccgcgcattctcctccggcatggctgcaaccgacatcctgttccgcatcatcctcaagccgggcgatcacatcgtcctcggcaacgatgcttacggcggaacctaccgcctgatcgacaccgtattcaccgcatggggcgtcgaatacaccgttgttgatacctccgtcgtggaagaggtcaaggcagcgatcaaggacaacaccaagctgatctgggtggaaaccccaaccaacccagcacttggcatcaccgacatcgaagcagtagcaaagctcaccgaaggcaccaacgccaagctggttgttgacaacaccttcgcatccccatacctgcagcagccactaaaactcggcgcacacgcagtcctgcactccaccaccaagtacatcggaggacactccgacgttgttggcggccttgtggttaccaacgaccaggaaatggacgaagaactgctgttcatgcagggcggcatcggaccgatcccatcagttttcgatgcatacctgaccgcccgtggcctcaagacccttgcagtgcgcatggatcgccactgcgacaacgcagaaaagatcgcggaattcctggactcccgcccagaggtctccaccgtgctctacccaggtctgaagaaccacccaggccacgaagtcgcagcgaagcagatgaagcgcttcggcggcatgatctccgtccgtttcgcaggcggcgaagaagcagctaagaagttctgtacctccaccaaactgatctgtctggccgagtccctcggtggcgtggaatccctcctggagcacccagcaaccatgacccaccagtcagctgccggctctcagctcgaggttccccgcgacctcgtgcgcatctccattggtattgaagacattgaagacctgctcgcagatgtcgagcaggccctcaataacctttag

SEQ ID NO: 12 - DNA, 18 bp, synthetic construct
  misc_feature 1..18: note = metB_N_del F
  source 1..18: mol_type = other DNA
ggcttcggagttggagcg

SEQ ID NO: 13 - DNA, 40 bp, synthetic construct
  misc_feature 1..40: note = metB_N_del R
  source 1..40: mol_type = other DNA
gccaaatagtttcccgggggtagatcaactcctgtaatca

SEQ ID NO: 14 - DNA, 40 bp, synthetic construct
  misc_feature 1..40: note = metB_C_del F
  source 1..40: mol_type = other DNA
caggagttgatctacccccgggaaactatttggcggcaag

SEQ ID NO: 15 - DNA, 19 bp, synthetic construct
  misc_feature 1..19: note = metB_C_del R
  source 1..19: mol_type = other DNA
tcgcgtctgggtgcgcatc

SEQ ID NO: 16 - DNA, 1314 bp, synthetic construct
  misc_feature 1..1314: note = Corynebacterium glutamicum metY
  source 1..1314: mol_type = other DNA
atgccaaagtacgacaattccaatgctgaccagtggggctttgaaacccgctccattcacgcaggccagtcagtagacgcacagaccagcgcacgaaaccttccgatctaccaatccaccgctttcgtgttcgactccgctgagcacgccaagcagcgtttcgcacttgaggatctaggccctgtttactcccgcctcaccaacccaaccgttgaggctttggaaaaccgcatcgcttccctcgaaggtggcgtccacgctgtagcgttctcctccggacaggccgcaaccaccaacgccattttgaacctggcaggagcgggcgaccacatcgtcacctccccacgcctctacggtggcaccgagactctattccttatcactcttaaccgcctgggtatcgatgtttccttcgtggaaaaccccgacgaccctgagtcctggcaggcagccgttcagccaaacaccaaagcattcttcggcgagactttcgccaacccacaggcagacgtcctggatattcctgcggtggctgaagttgcgcaccgcaacagcgttccactgatcatcgacaacaccatcgctaccgcagcgctcgtgcgcccgctcgagctcggcgcagacgttgtcgtcgcttccctcaccaagttctacaccggcaacggctccggactgggcggcgtgcttatcgacggcggaaagttcgattggactgtcgaaaaggatggaaagccagtattcccctacttcgtcactccagatgctgcttaccacggattgaagtacgcagaccttggtgcaccagccttcggcctcaaggttcgcgttggccttctacgcgacaccggctccaccctctccgcattcaacgcatgggctgcagtccagggcatcgacaccctttccctgcgcctggagcgccacaacgaaaacgccatcaaggttgcagaattcctcaacaaccacgagaaggtggaaaaggttaacttcgcaggcctgaaggattccccttggtacgcaaccaaggaaaagcttggcctgaagtacaccggctccgttctcaccttcgagatcaagggcggcaaggatgaggcttgggcatttatcgacgccctgaagctacactccaaccttgcaaacatcggcgatgttcgctccctcgttgttcacccagcaaccaccacccattcacagtccgacgaagctggcctggcacgcgcgggcgttacccagtccaccgtccgcctgtccgttggcatcgagaccattgatgatatcatcgctgacctcgaaggcggctttgctgcaatctag

SEQ ID NO: 17 - DNA, 18 bp, synthetic construct
  misc_feature 1..18: note = metY_N_del F
  source 1..18: mol_type = other DNA
ccaaagacaaggagacca

SEQ ID NO: 18 - DNA, 40 bp, synthetic construct
  misc_feature 1..40: note = metY_N_del R
  source 1..40: mol_type = other DNA
agtctatttaaagcccgggttggaggtccttaagagtttt

SEQ ID NO: 19 - DNA, 40 bp, synthetic construct
  misc_feature 1..40: note = metY_C_del F
  source 1..40: mol_type = other DNA
taaggacctccaacccgggctttaaatagactcaccccag

SEQ ID NO: 20 - DNA, 18 bp, synthetic construct
  misc_feature 1..18: note = metY_C_del R
  source 1..18: mol_type = other DNA
atgccgagtgcgtcgagg

SEQ ID NO: 21 - DNA, 1266 bp, unidentified
  misc_feature 1..1266: note = Corynebacterium glutamicum lysC
  source 1..1266: mol_type = genomic DNA
gtggccctggtcgtacagaaatatggcggttcctcgcttgagagtgcggaacgcattagaaacgtcgctgaacggatcgttgccaccaagaaggctggaaatgatgtcgtggttgtctgctccgcaatgggagacaccacggatgaacttctagaacttgcagcggcagtgaatcccgttccgccagctcgtgaaatggatatgctcctgactgctggtgagcgtatttctaacgctctcgtcgccatggctattgagtcccttggcgcagaagcccaatctttcacgggctctcaggctggtgtgctcaccaccgagcgccacggaaacgcacgcattgttgatgtcactccaggtcgtgtgcgtgaagcactcgatgagggcaagatctgcattgttgctggtttccagggtgttaataaagaaacccgcgatgtcaccacgttgggtcgtggtggttctgacaccactgcagttgcgttggcagctgctttgaacgctgatgtgtgtgagatttactcggacgttgacggtgtgtataccgctgacccgcgcatcgttcctaatgcacagaagctggaaaagctcagcttcgaagaaatgctggaacttgctgctgttggctccaagattttggtgctgcgcagtgttgaatacgctcgtgcattcaatgtgccacttcgcgtacgctcgtcttatagtaatgatcccggcactttgattgccggctctatggaggatattcctgtggaagaagcagtccttaccggtgtcgcaaccgacaagtccgaagccaaagtaaccgttctgggtatttccgataagccaggcgaggctgcgaaggttttccgtgcgttggctgatgcagaaatcaacattgacatggttctgcagaacgtctcttctgtagaagacggcaccaccgacatcaccttcacctgccctcgttccgacggccgccgcgcgatggagatcttgaagaagcttcaggttcagggcaactggaccaatgtgctttacgacgaccaggtcggcaaagtctccctcgtgggtgctggcatgaagtctcacccaggtgttaccgcagagttcatggaagctctgcgcgatgtcaacgtgaacatcgaattgatttccacctctgagattcgtatttccgtgctgatccgtgaagatgatctggatgctgctgcacgtgcattgcatgagcagttccagctgggcggcgaagacgaagccgtcgtttatgcaggcaccggacgctaa

SEQ ID NO: 22 - DNA, 19 bp, synthetic construct
  misc_feature 1..19: note = lysC_L377K_5 F
  source 1..19: mol_type = other DNA
cagaagctggaaaagctca

SEQ ID NO: 23 - DNA, 40 bp, synthetic construct
  misc_feature 1..40: note = lysC_L377K_5 R
  source 1..40: mol_type = other DNA
atctcagaggtggaaatcttttcgatgttcacgttgacat

SEQ ID NO: 24 - DNA, 40 bp, synthetic construct
  misc_feature 1..40: note = lysC_L377K_3 F
  source 1..40: mol_type = other DNA
tgtcaacgtgaacatcgaaaagatttccacctctgagatt

SEQ ID NO: 25 - DNA, 19 bp, synthetic construct
  misc_feature 1..19: note = lysC_L377K_3 R
  source 1..19: mol_type = other DNA
tccttgtcggaagggttca

SEQ ID NO: 26 - DNA, 1134 bp, synthetic construct
  misc_feature 1..1134: note = Corynebacterium glutamicum metX
  source 1..1134: mol_type = other DNA
atgcccaccctcgcgccttcaggtcaacttgaaatccaagcgatcggtgatgtctccaccgaagccggagcaatcattacaaacgctgaaatcgcctatcaccgctggggtgaataccgcgtagataaagaaggacgcagcaatgtcgttctcatcgaacacgccctcactggagattccaacgcagccgattggtgggctgacttgctcggtcccggcaaagccatcaacactgatatttactgcgtgatctgtaccaacgtcatcggtggttgcaacggttccaccggacctggctccatgcatccagatggaaatttctggggtaatcgcttccccgccacgtccattcgtgatcaggtaaacgccgaaaaacaattcctcgacgcactcggcatcaccacggtcgccgcagtacttggtggttccatgggtggtgcccgcaccctagagtgggccgcaatgtacccagaaactgttggcgcagctgctgttcttgcagtttctgcacgcgccagcgcctggcaaatcggcattcaatccgcccaaattaaggcgattgaaaacgaccaccactggcacgaaggcaactactacgaatccggctgcaacccagccaccggactcggcgccgcccgacgcatcgcccacctcacctaccgtggcgaactagaaatcgacgaacgcttcggcaccaaagcccaaaagaacgaaaacccactcggtccctaccgcaagcccgaccagcgcttcgccgtggaatcctacttggactaccaagcagacaagctagtacagcgtttcgacgccggctcctacgtcttgctcaccgacgccctcaaccgccacgacattggtcgcgaccgcggaggcctcaacaaggcactcgaatccatcaaagttccagtccttgtcgcaggcgtagataccgatattttgtacccctaccaccagcaagaacacctctccagaaacctgggaaatctactggcaatggcaaaaatcgtatcccctgtcggccacgatgctttcctcaccgaaagccgccaaatggatcgcatcgtgaggaacttcttcagcctcatctccccagacgaagacaacccttcgacctacatcgagttctacatctaa

SEQ ID NO: 27 - DNA, 28 bp, synthetic construct
  misc_feature 1..28: note = metX F
  source 1..28: mol_type = other DNA
ggatcccctcgttgttcacccagcaacc

SEQ ID NO: 28 - DNA, 30 bp, synthetic construct
  misc_feature 1..30: note = metX R
  source 1..30: mol_type = other DNA
ggatcccaaagtcacaactacttatgttag